European Patent Application EP 4 134 431 A1, published February 15, 2023. Title: Genome modification method and genome modification Kit. Applicant: Logomix, Inc. Tokyo Institute of Technology. The sequence listing filed with the application follows.

SEQUENCE LISTING (73 sequences)

SEQ ID NO: 1 - protein, 1423 aa, Staphylococcus pyogenes
MDYKDHDGDYKDHDIDYKDDDDKMAPKKKRKVGIHGVPAADKKYSIGLDIGTNSVGWAVITDEYKVPSKKFKVLGNTDRHSIKKNLIGALLFDSGETAEATRLKRTARRRYTRRKNRICYLQEIFSNEMAKVDDSFFHRLEESFLVEEDKKHERHPIFGNIVDEVAYHEKYPTIYHLRKKLVDSTDKADLRLIYLALAHMIKFRGHFLIEGDLNPDNSDVDKLFIQLVQTYNQLFEENPINASGVDAKAILSARLSKSRRLENLIAQLPGEKKNGLFGNLIALSLGLTPNFKSNFDLAEDAKLQLSKDTYDDDLDNLLAQIGDQYADLFLAAKNLSDAILLSDILRVNTEITKAPLSASMIKRYDEHHQDLTLLKALVRQQLPEKYKEIFFDQSKNGYAGYIDGGASQEEFYKFIKPILEKMDGTEELLVKLNREDLLRKQRTFDNGSIPHQIHLGELHAILRRQEDFYPFLKDNREKIEKILTFRIPYYVGPLARGNSRFAWMTRKSEETITPWNFEEVVDKGASAQSFIERMTNFDKNLPNEKVLPKHSLLYEYFTVYNELTKVKYVTEGMRKPAFLSGEQKKAIVDLLFKTNRKVTVKQLKEDYFKKIECFDSVEISGVEDRFNASLGTYHDLLKIIKDKDFLDNEENEDILEDIVLTLTLFEDREMIEERLKTYAHLFDDKVMKQLKRRRYTGWGRLSRKLINGIRDKQSGKTILDFLKSDGFANRNFMQLIHDDSLTFKEDIQKAQVSGQGDSLHEHIANLAGSPAIKKGILQTVKVVDELVKVMGRHKPENIVIEMARENQTTQKGQKNSRERMKRIEEGIKELGSQILKEHPVENTQLQNEKLYLYYLQNGRDMYVDQELDINRLSDYDVDHIVPQSFLKDDSIDNKVLTRSDKNRGKSDNVPSEEVVKKMKNYWRQLLNAKLITQRKFDNLTKAERGGLSELDKAGFIKRQLVETRQITKHVAQILDSRMNTKYDENDKLIREVKVITLKSKLVSDFRKDFQFYKVREINNYHHAHDAYLNAVVGTALIKKYPKLESEFVYGDYKVYDVRKMIAKSEQEIGKATAKYFFYSNIMNFFKTEITLANGEIRKRPLIETNGETGEIVWDKGRDFATVRKVLSMPQVNIVKKTEVQTGGFSKESILPKRNSDKLIARKKDWDPKKYGGFDSPTVAYSVLVVAKVEKGKSKKLKSVKELLGITIMERSSFEKNPIDFLEAKGYKEVKKDLIIKLPKYSLFELENGRKRMLASAGELQKGNELALPSKYVNFLYLASHYEKLKGSPEDNEQKQLFVEQHKHYLDEIIEQISEFSKRVILADANLDKVLSAYNKHRDKPIREQAENIIHLFTLTNLGAPAAFKYFDTTIDRKRYTSTKEVLDATLIHQSITGLYETRIDLSQLGGDKRPAATKKAGQAKKKK

SEQ ID NO: 2 - DNA, 810 bp, Homo sapiens
ttccccagaggtatcttccatggcttttccagaccccaactctggcccgttcgcttcttcttcagaaaggctcccgtttgcttcttctgcaggaaggcttgtattttcagaaagttcttgctcctcgattcgaggactcaactcactaggggaaccaaactctgtttccaggggagtggagagagaaactgggtccccctcccgtagctcctgggacacagctgagccagccacaggatctggggacaaccggggcggatcccccctttcgggaggcggtggcatcagttcagagtccgcatttttattcatcggggaagcgtggggagaaggatgggctggagctgggtcctggtctgaaggacagcagtccggagctaacggttgagtctccaaagtcttcatactgcagaggaagcacagcggagattagcctcagccaggatggcttcgaagttctcagggatccgacgcagagctaaagaaacccacctgtgcttccctcctcttctgggagtaggcagaagactcccgggaggagaggcgaacagcggacgccaattcttttgaaagcactgtgttccttagcaccgcgggtcgctacgggcctcttgctgtcgcgggatttcggtccaccttccgattgggccgccgcatcccggatcagatttcgcgggcgacccacggaacccgcggagccgggacgtgaaaggttagaaggtttcccgttcccatcaagccctagggctcctcgtggctgctgggagttgtagtctgaacgcttctatcttggcgagaagcgcctacgct

SEQ ID NO: 3 - DNA, 792 bp, Homo sapiens
ctgagtcaggaaacattttcagacctatggaaactgtgagtggatccattggaagggcaggcccaccaccccgaccccaaccccagccccctagcagagacctgtgggaagcgaaaattccatgggactgactttctgctcttgtctttcagacttcctgaaaacaacgttctggtaaggacaagggttgggctggggacctggagggctggggggctggggggctgaggacctggtcctctgactgctcttttcacccatctacagtcccccttgccgtcccaagcaatggatgatttgatgctgtccccggacgatattgaacaatggttcactgaagacccaggtccagatgaagctcccagaatgccagaggctgctccccccgtggcccctgcaccagcagctcctacaccggcggcccctgcaccagccccctcctggcccctgtcatcttctgtcccttcccagaaaacctaccagggcagctacggtttccgtctgggcttcttgcattctgggacagccaagtctgtgacttgcacggtcagttgccctgaggggctggcttccatgagacttcaatgcctggccgtatccccctgcatttcttttgtttggaactttgggattcctcttcaccctttggcttcctgtcagtgtttttttatagtttacccacttaatgtgtgatctctgactcctgtcccaaagttgaatattccccccttgaatttgggcttttatccatcccatcacaccctcagcatctctcctggggatgcagaactt

SEQ ID NO: 4 - DNA, 23 bp, Artificial sequence
  taget sequence for gRNA
ctcagagggggctcgacgctagg

SEQ ID NO: 5 - DNA, 20 bp, Artificial sequence
  primer sequence
tgccccgttgttatccttac

SEQ ID NO: 6 - DNA, 20 bp, Artificial sequence
  primer sequence
gctcgtagaaggggaggttg

SEQ ID NO: 7 - DNA, 19 bp, Artificial sequence
  primer sequence
gtcaccgagctgcaagaac

SEQ ID NO: 8 - DNA, 20 bp, Artificial sequence
  primer sequence
gaagacggcagcaaagaaac

SEQ ID NO: 9 - DNA, 20 bp, Artificial sequence
  primer sequence
tgccccgttgttatccttac

SEQ ID NO: 10 - DNA, 22 bp, Artificial sequence
  primer sequence
gcttcaatatgtactgccgaaa

SEQ ID NO: 11 - DNA, 20 bp, Artificial sequence
  primer sequence
gaagccattgcgattggtag

SEQ ID NO: 12 - DNA, 20 bp, Artificial sequence
  primer sequence
gaagacggcagcaaagaaac

SEQ ID NO: 13 - DNA, 23 bp, Artificial sequence
  taget sequence for gRNA
ggcgcaacgcgatcgcgtaaggg

SEQ ID NO: 14 - DNA, 20 bp, Artificial sequence
  primer sequence
tgccccgttgttatccttac

SEQ ID NO: 15 - DNA, 20 bp, Artificial sequence
  primer sequence
gaagacggcagcaaagaaac

SEQ ID NO: 16 - RNA, 20 nt, Artificial Sequence
  gRNA for upstream region of human TP53
cucagagggggcucgacgcu

SEQ ID NO: 17 - RNA, 20 nt, Artificial Sequence
  gRNA for downstream of human TP53
ggugcuuuaagaauuaccgc

SEQ ID NO: 18 - RNA, 20 nt, Artificial Sequence
  gRNA for upstream region of MLH1
gcgccugacgucgcguucgc

SEQ ID NO: 19 - RNA, 20 nt, Artificial Sequence
  gRNA for downstream region of MLH1
ggaggccuuggcacggguuc

SEQ ID NO: 20 - RNA, 20 nt, Artificial Sequence
  gRNA for upstream region of human CD44
cgaggauggcggaccgaacc

SEQ ID NO: 21 - RNA, 20 nt, Artificial Sequence
  gRNA for downstream region of human CD44
gccaaguggacucaacggag

SEQ ID NO: 22 - RNA, 20 nt, Artificial Sequence
  gRNA for upstream region of human MET
gggccgcgcgcgccgaugcc

SEQ ID NO: 23 - RNA, 20 nt, Artificial Sequence
  gRNA for downstream region of MET
guucccaccucgcaagcaau

SEQ ID NO: 24 - RNA, 20 nt, Artificial Sequence
  gRNA for upsteam region of APP
cucccgggggugucguauaa

SEQ ID NO: 25 - RNA, 20 nt, Artificial Sequence
  gRNA for downstream region of APP
uucuauaaauggacaccgau

SEQ ID NO: 26 - DNA, 20 bp, Artificial Sequence
  Forward primer for MLH1 5' junction PCR
ccaagaacgcttccatttct

SEQ ID NO: 27 - DNA, 18 bp, Artificial Sequence
  Reverse primer for MLH1 5' junction PCR
ccctgtgcctggtctgtc

SEQ ID NO: 28 - DNA, 20 bp, Artificial Sequence
  Forward primer for MLH1 3' junction PCR
ttctgaggtctccagcaagt

SEQ ID NO: 29 - DNA, 24 bp, Artificial Sequence
  Reverse primer for MLH1 3' junction PCR
aagttgaagatgaattgaaagcag

SEQ ID NO: 30 - DNA, 20 bp, Artificial Sequence
  Forward primer for Puromycin 5' junction PCR
ccaagaacgcttccatttct

SEQ ID NO: 31 - DNA, 20 bp, Artificial Sequence
  Reverse primer for Puromycin 5' junction PCR
gctcgtagaaggggaggttg

SEQ ID NO: 32 - DNA, 19 bp, Artificial Sequence
  Forward primer for Puromycin 3' junction PCR
gtcaccgagctgcaagaac

SEQ ID NO: 33 - DNA, 24 bp, Artificial Sequence
  Reverse primer for Puromycin 3' junction PCR
aagttgaagatgaattgaaagcag

SEQ ID NO: 34 - DNA, 20 bp, Artificial Sequence
  Forward primer for Blasticidin 5' junction PCR
ccaagaacgcttccatttct

SEQ ID NO: 35 - DNA, 22 bp, Artificial Sequence
  Reverse primer for Blasticidin 5' junction PCR
gcttcaatatgtactgccgaaa

SEQ ID NO: 36 - DNA, 20 bp, Artificial Sequence
  Forward primer for Blasticidin 3' junction PCR
gaagccattgcgattggtag

SEQ ID NO: 37 - DNA, 24 bp, Artificial Sequence
  Reverse primer for Blasticidin 3' junction PCR
aagttgaagatgaattgaaagcag

SEQ ID NO: 38 - DNA, 20 bp, Artificial Sequence
  Forward primer for CD44 5' junction PCR
agtggatggacaggaggatg

SEQ ID NO: 39 - DNA, 18 bp, Artificial Sequence
  Reverse primer for CD44 5' junction PCR
gcgaaaggagctggagga

SEQ ID NO: 40 - DNA, 20 bp, Artificial Sequence
  Forward primer for CD443' junction PCR
atggagctgtggaggacaga

SEQ ID NO: 41 - DNA, 20 bp, Artificial Sequence
  Reverse primer for CD443' junction PCR
gagtgggtctgagtgggaac

SEQ ID NO: 42 - DNA, 20 bp, Artificial Sequence
  Forward primer for Puromycin 5' junction PCR-2
agtggatggacaggaggatg

SEQ ID NO: 43 - DNA, 20 bp, Artificial Sequence
  Reverse primer for Puromycin 5' junction PCR-2
gctcgtagaaggggaggttg

SEQ ID NO: 44 - DNA, 19 bp, Artificial Sequence
  Forward primer for Puromycin 3' junction PCR-2
gtcaccgagctgcaagaac

SEQ ID NO: 45 - DNA, 20 bp, Artificial Sequence
  Reverse primer for Puromycin 3' junction PCR-2
gagtgggtctgagtgggaac

SEQ ID NO: 46 - DNA, 20 bp, Artificial Sequence
  Forward primer for Blasticidin 5' junction PCR-2
agtggatggacaggaggatg

SEQ ID NO: 47 - DNA, 22 bp, Artificial Sequence
  Reverse primer for Blasticidin 5' junction PCR-2
gcttcaatatgtactgccgaaa

SEQ ID NO: 48 - DNA, 20 bp, Artificial Sequence
  Forward primer for Blasticidin 3' junction PCR-2
gaagccattgcgattggtag

SEQ ID NO: 49 - DNA, 20 bp, Artificial Sequence
  Reverse primer for Blasticidin 3' junction PCR-2
gagtgggtctgagtgggaac

SEQ ID NO: 50 - DNA, 26 bp, Artificial Sequence
  Forward primer for MET 5' junction PCR
tgaaatcactcttatgtaacctctgg

SEQ ID NO: 51 - DNA, 20 bp, Artificial Sequence
  Reverse primer for MET 5' junction PCR
aaggggctgcaattttacct

SEQ ID NO: 52 - DNA, 20 bp, Artificial Sequence
  Forward primer for MET 3' junction PCR
gggtggatggattgaaaaga

SEQ ID NO: 53 - DNA, 22 bp, Artificial Sequence
  Reverse primer for MET 3' junction PCR
tgcaggtataggcagtgacaag

SEQ ID NO: 54 - DNA, 26 bp, Artificial Sequence
  Forward primer for Puromycin 5' junction PCR-3
tgaaatcactcttatgtaacctctgg

SEQ ID NO: 55 - DNA, 20 bp, Artificial Sequence
  Reverse primer for Puromycin 5' junction PCR-3
gctcgtagaaggggaggttg

SEQ ID NO: 56 - DNA, 19 bp, Artificial Sequence
  Forward primer for Puromycin 3' junction PCR-3
gtcaccgagctgcaagaac

SEQ ID NO: 57 - DNA, 22 bp, Artificial Sequence
  Reverse primer for Puromycin 3' junction PCR-3
tgcaggtataggcagtgacaag

SEQ ID NO: 58 - DNA, 26 bp, Artificial Sequence
  Forward primer for Blasticidin 5' junction PCR-3
tgaaatcactcttatgtaacctctgg

SEQ ID NO: 59 - DNA, 22 bp, Artificial Sequence
  Reverse primer for Blasticidin 5' junction PCR-3
gcttcaatatgtactgccgaaa

SEQ ID NO: 60 - DNA, 20 bp, Artificial Sequence
  Forward primer for Blasticidin 3' junction PCR-3
gaagccattgcgattggtag

SEQ ID NO: 61 - DNA, 22 bp, Artificial Sequence
  Reverse primer for Blasticidin 3' junction PCR-3
tgcaggtataggcagtgacaag

SEQ ID NO: 62 - DNA, 20 bp, Artificial Sequence
  Forward primer for APP 5' junction PCR
ggggagctggtacagaaatg

SEQ ID NO: 63 - DNA, 20 bp, Artificial Sequence
  Reverse primer for APP 5' junction PCR
caggatcagggaaaggtgag

SEQ ID NO: 64 - DNA, 20 bp, Artificial Sequence
  Forward primer for APP 3' junction PCR
gaacggctacgaaaatccaa

SEQ ID NO: 65 - DNA, 19 bp, Artificial Sequence
  Reverse primer for APP 3' junction PCR
ctcttctccccacccaaaa

SEQ ID NO: 66 - DNA, 20 bp, Artificial Sequence
  Forward primer for Puromycin 5' junction PCR-4
ggggagctggtacagaaatg

SEQ ID NO: 67 - DNA, 20 bp, Artificial Sequence
  Reverse primer for Puromycin 5' junction PCR-4
gctcgtagaaggggaggttg

SEQ ID NO: 68 - DNA, 19 bp, Artificial Sequence
  Forward primer for Puromycin 3' junction PCR-4
gtcaccgagctgcaagaac

SEQ ID NO: 69 - DNA, 19 bp, Artificial Sequence
  Reverse primer for Puromycin 3' junction PCR-4
ctcttctccccacccaaaa

SEQ ID NO: 70 - DNA, 20 bp, Artificial Sequence
  Forward primer for Blasticidin 5' junction PCR-4
ggggagctggtacagaaatg

SEQ ID NO: 71 - DNA, 22 bp, Artificial Sequence
  Reverse primer for Blasticidin 5' junction PCR-4
gcttcaatatgtactgccgaaa

SEQ ID NO: 72 - DNA, 20 bp, Artificial Sequence
  Forward primer for Blasticidin 3' junction PCR-4
gaagccattgcgattggtag

SEQ ID NO: 73 - DNA, 19 bp, Artificial Sequence
  Reverse primer for Blasticidin 3' junction PCR-4
ctcttctccccacccaaaa